European Patent Application EP 4 755 910 A1, published June 10, 2026. Title: 抗白介素-11抗体在制备肿瘤治疗药物中的应用. Applicant: 迈威（上海）生物科技股份有限公司. The sequence listing filed with the application follows.

SEQUENCE LISTING (44 sequences)

SEQ ID NO: 1 - protein, 120 aa, synthetic construct
EVQLVESGGGLVQPGGSLRLSCAASGFTFSSFGMHWVRQAPGKGLEWVAYITPGSNTIYYADTVKGRFTISRDNAKNSLYLQMNSLRAEDTAVYYCAREYYSYDEGFAYWGQGTLVTVSS

SEQ ID NO: 2 - protein, 108 aa, synthetic construct
EIVLTQSPATLSLSPGERATLSCSVSDLIPSQYLHWYQQKPGQAPRLLIYRTSNLASGIPARFSGSGSGTDFTLTISSLEPEDFAVYYCQQGVDVPFTFGQGTKLEIK

SEQ ID NO: 3 - protein, 120 aa, synthetic construct
EVQLVESGGGLVQPGGSLRLSCAASGFTFSSFGMHWVRQAPGKGLEWVAYITPGSNTIYYADTVKGRFTISRDNAKNSLYLQMNSLRAEDTAVYYCAREYYSYDEGFASWGQGTLVTVSS

SEQ ID NO: 4 - protein, 108 aa, synthetic construct
EIVLTQSPATLSLSPGERATLSCSVSDLIPSQYLHWYQQKPGQAPRLLIYDASNLASGIPARFSGSGSGTDFTLTISSLEPEDFAVYYCQQGVDVPFTFGQGTKLEIK

SEQ ID NO: 5 - protein, 117 aa, synthetic construct
EVQLVQSGAEVKKPGASVKVSCKASGYTFTHYNMDWVRQAPGQGLEWMGTIYPGNADTSYNQKFKGRVTMTRDTSTSTVYMELSSLRSEDTAVYYCARGDLYALDYWGQGTLVTVSS

SEQ ID NO: 6 - protein, 107 aa, synthetic construct
DIQMTQSPSSLSASVGDRVTITCKASQSVYRDVAWYQQKPGKAPKLLIYSASNRYTGVPSRFSGSGSGTDFTFTISSLQPEDIATYYCQHDYSSPYTFGQGTKLEIK

SEQ ID NO: 7 - protein, 120 aa, synthetic construct
EVQLVESGGGLVQPGGSLRLSCAASGFTFSSFGMHWVRQAPGKGLEWVAYITPGSNTIYYADTVKGRFTISRDNAKNSLYLQMNSLRAEDTAVYYCAREYSSYDEGFAYWGQGTLVTVSS

SEQ ID NO: 8 - protein, 108 aa, synthetic construct; identical to SEQ ID NO: 4

SEQ ID NO: 9 - protein, 117 aa, synthetic construct
EVQLVQSGAEVKKPGASVKVSCKASGYTFTTYNMDWVRQAPGQGLEWMGTIYPGNGDTSYNQKFKGRVTMTRDTSTSTVYMELSSLRSEDTAVYYCARGDLYALDYWGQGTLVTVSS

SEQ ID NO: 10 - protein, 107 aa, synthetic construct
DIQMTQSPSSLSASVGDRVTITCKASQSVSNDVAWYQQKPGKAPKLLIYSASNRYTGVPSRFSGSGSGTDFTFTISSLQPEDIATYYCQHDYSSPYTFGQGTKLEIK

SEQ ID NO: 11 - protein, 117 aa, synthetic construct
EVQLVQSGAEVKKPGASVKVSCKASGYTFNHYDMDWVRQAPGQGLEWMGTIYPGNGDTSYNQKFKGRVTMTRDTSTSTVYMELSSLRSEDTAVYYCARGDLYALDYWGQGTLVTVSS

SEQ ID NO: 12 - protein, 107 aa, synthetic construct; identical to SEQ ID NO: 6

SEQ ID NO: 13 - protein, 450 aa, synthetic construct
EVQLVESGGGLVQPGGSLRLSCAASGFTFSSFGMHWVRQAPGKGLEWVAYITPGSNTIYYADTVKGRFTISRDNAKNSLYLQMNSLRAEDTAVYYCAREYYSYDEGFAYWGQGTLVTVSSASTKGPSVFPLAPSSKSTSGGTAALGCLVKDYFPEPVTVSWNSGALTSGVHTFPAVLQSSGLYSLSSVVTVPSSSLGTQTYICNVNHKPSNTKVDKKVEPKSCDKTHTCPPCPAPELLGGPSVFLFPPKPKDTLMISRTPEVTCVVVDVSHEDPEVKFNWYVDGVEVHNAKTKPREEQYNSTYRVVSVLTVLHQDWLNGKEYKCKVSNKALPAPIEKTISKAKGQPREPQVYTLPPSRDELTKNQVSLTCLVKGFYPSDIAVEWESNGQPENNYKTTPPVLDSDGSFFLYSKLTVDKSRWQQGNVFSCSVMHEALHNHYTQKSLSLSPGK

SEQ ID NO: 14 - protein, 215 aa, synthetic construct
EIVLTQSPATLSLSPGERATLSCSVSDLIPSQYLHWYQQKPGQAPRLLIYRTSNLASGIPARFSGSGSGTDFTLTISSLEPEDFAVYYCQQGVDVPFTFGQGTKLEIKRTVAAPSVFIFPPSDEQLKSGTASVVCLLNNFYPREAKVQWKVDNALQSGNSQESVTEQDSKDSTYSLSSTLTLSKADYEKHKVYACEVTHQGLSSPVTKSFNRGEC

SEQ ID NO: 15 - protein, 450 aa, synthetic construct
EVQLVESGGGLVQPGGSLRLSCAASGFTFSSFGMHWVRQAPGKGLEWVAYITPGSNTIYYADTVKGRFTISRDNAKNSLYLQMNSLRAEDTAVYYCAREYYSYDEGFASWGQGTLVTVSSASTKGPSVFPLAPSSKSTSGGTAALGCLVKDYFPEPVTVSWNSGALTSGVHTFPAVLQSSGLYSLSSVVTVPSSSLGTQTYICNVNHKPSNTKVDKKVEPKSCDKTHTCPPCPAPELLGGPSVFLFPPKPKDTLMISRTPEVTCVVVDVSHEDPEVKFNWYVDGVEVHNAKTKPREEQYNSTYRVVSVLTVLHQDWLNGKEYKCKVSNKALPAPIEKTISKAKGQPREPQVYTLPPSRDELTKNQVSLTCLVKGFYPSDIAVEWESNGQPENNYKTTPPVLDSDGSFFLYSKLTVDKSRWQQGNVFSCSVMHEALHNHYTQKSLSLSPGK

SEQ ID NO: 16 - protein, 215 aa, synthetic construct
EIVLTQSPATLSLSPGERATLSCSVSDLIPSQYLHWYQQKPGQAPRLLIYDASNLASGIPARFSGSGSGTDFTLTISSLEPEDFAVYYCQQGVDVPFTFGQGTKLEIKRTVAAPSVFIFPPSDEQLKSGTASVVCLLNNFYPREAKVQWKVDNALQSGNSQESVTEQDSKDSTYSLSSTLTLSKADYEKHKVYACEVTHQGLSSPVTKSFNRGEC

SEQ ID NO: 17 - protein, 447 aa, synthetic construct
EVQLVQSGAEVKKPGASVKVSCKASGYTFTHYNMDWVRQAPGQGLEWMGTIYPGNADTSYNQKFKGRVTMTRDTSTSTVYMELSSLRSEDTAVYYCARGDLYALDYWGQGTLVTVSSASTKGPSVFPLAPSSKSTSGGTAALGCLVKDYFPEPVTVSWNSGALTSGVHTFPAVLQSSGLYSLSSVVTVPSSSLGTQTYICNVNHKPSNTKVDKKVEPKSCDKTHTCPPCPAPELLGGPSVFLFPPKPKDTLMISRTPEVTCVVVDVSHEDPEVKFNWYVDGVEVHNAKTKPREEQYNSTYRVVSVLTVLHQDWLNGKEYKCKVSNKALPAPIEKTISKAKGQPREPQVYTLPPSRDELTKNQVSLTCLVKGFYPSDIAVEWESNGQPENNYKTTPPVLDSDGSFFLYSKLTVDKSRWQQGNVFSCSVMHEALHNHYTQKSLSLSPGK

SEQ ID NO: 18 - protein, 214 aa, synthetic construct
DIQMTQSPSSLSASVGDRVTITCKASQSVYRDVAWYQQKPGKAPKLLIYSASNRYTGVPSRFSGSGSGTDFTFTISSLQPEDIATYYCQHDYSSPYTFGQGTKLEIKRTVAAPSVFIFPPSDEQLKSGTASVVCLLNNFYPREAKVQWKVDNALQSGNSQESVTEQDSKDSTYSLSSTLTLSKADYEKHKVYACEVTHQGLSSPVTKSFNRGEC

SEQ ID NO: 19 - protein, 450 aa, synthetic construct
EVQLVESGGGLVQPGGSLRLSCAASGFTFSSFGMHWVRQAPGKGLEWVAYITPGSNTIYYADTVKGRFTISRDNAKNSLYLQMNSLRAEDTAVYYCAREYSSYDEGFAYWGQGTLVTVSSASTKGPSVFPLAPSSKSTSGGTAALGCLVKDYFPEPVTVSWNSGALTSGVHTFPAVLQSSGLYSLSSVVTVPSSSLGTQTYICNVNHKPSNTKVDKKVEPKSCDKTHTCPPCPAPELLGGPSVFLFPPKPKDTLMISRTPEVTCVVVDVSHEDPEVKFNWYVDGVEVHNAKTKPREEQYNSTYRVVSVLTVLHQDWLNGKEYKCKVSNKALPAPIEKTISKAKGQPREPQVYTLPPSRDELTKNQVSLTCLVKGFYPSDIAVEWESNGQPENNYKTTPPVLDSDGSFFLYSKLTVDKSRWQQGNVFSCSVMHEALHNHYTQKSLSLSPGK

SEQ ID NO: 20 - protein, 215 aa, synthetic construct; identical to SEQ ID NO: 16

SEQ ID NO: 21 - protein, 447 aa, synthetic construct
EVQLVQSGAEVKKPGASVKVSCKASGYTFTTYNMDWVRQAPGQGLEWMGTIYPGNGDTSYNQKFKGRVTMTRDTSTSTVYMELSSLRSEDTAVYYCARGDLYALDYWGQGTLVTVSSASTKGPSVFPLAPSSKSTSGGTAALGCLVKDYFPEPVTVSWNSGALTSGVHTFPAVLQSSGLYSLSSVVTVPSSSLGTQTYICNVNHKPSNTKVDKKVEPKSCDKTHTCPPCPAPELLGGPSVFLFPPKPKDTLMISRTPEVTCVVVDVSHEDPEVKFNWYVDGVEVHNAKTKPREEQYNSTYRVVSVLTVLHQDWLNGKEYKCKVSNKALPAPIEKTISKAKGQPREPQVYTLPPSRDELTKNQVSLTCLVKGFYPSDIAVEWESNGQPENNYKTTPPVLDSDGSFFLYSKLTVDKSRWQQGNVFSCSVMHEALHNHYTQKSLSLSPGK

SEQ ID NO: 22 - protein, 214 aa, synthetic construct
DIQMTQSPSSLSASVGDRVTITCKASQSVSNDVAWYQQKPGKAPKLLIYSASNRYTGVPSRFSGSGSGTDFTFTISSLQPEDIATYYCQHDYSSPYTFGQGTKLEIKRTVAAPSVFIFPPSDEQLKSGTASVVCLLNNFYPREAKVQWKVDNALQSGNSQESVTEQDSKDSTYSLSSTLTLSKADYEKHKVYACEVTHQGLSSPVTKSFNRGEC

SEQ ID NO: 23 - protein, 447 aa, synthetic construct
EVQLVQSGAEVKKPGASVKVSCKASGYTFNHYDMDWVRQAPGQGLEWMGTIYPGNGDTSYNQKFKGRVTMTRDTSTSTVYMELSSLRSEDTAVYYCARGDLYALDYWGQGTLVTVSSASTKGPSVFPLAPSSKSTSGGTAALGCLVKDYFPEPVTVSWNSGALTSGVHTFPAVLQSSGLYSLSSVVTVPSSSLGTQTYICNVNHKPSNTKVDKKVEPKSCDKTHTCPPCPAPELLGGPSVFLFPPKPKDTLMISRTPEVTCVVVDVSHEDPEVKFNWYVDGVEVHNAKTKPREEQYNSTYRVVSVLTVLHQDWLNGKEYKCKVSNKALPAPIEKTISKAKGQPREPQVYTLPPSRDELTKNQVSLTCLVKGFYPSDIAVEWESNGQPENNYKTTPPVLDSDGSFFLYSKLTVDKSRWQQGNVFSCSVMHEALHNHYTQKSLSLSPGK

SEQ ID NO: 24 - protein, 214 aa, synthetic construct; identical to SEQ ID NO: 18

SEQ ID NO: 25 - protein, 330 aa, synthetic construct
ASTKGPSVFPLAPSSKSTSGGTAALGCLVKDYFPEPVTVSWNSGALTSGVHTFPAVLQSSGLYSLSSVVTVPSSSLGTQTYICNVNHKPSNTKVDKKVEPKSCDKTHTCPPCPAPEAAGGPSVFLFPPKPKDTLMISRTPEVTCVVVDVSHEDPEVKFNWYVDGVEVHNAKTKPREEQYNSTYRVVSVLTVLHQDWLNGKEYKCKVSNKALPAPIEKTISKAKGQPREPQVYTLPPSRDELTKNQVSLTCLVKGFYPSDIAVEWESNGQPENNYKTTPPVLDSDGSFFLYSKLTVDKSRWQQGNVFSCSVMHEALHNHYTQKSLSLSPGK

SEQ ID NO: 26 - protein, 5 aa, synthetic construct
SFGMH

SEQ ID NO: 27 - protein, 17 aa, synthetic construct
YITPGSNTIYYADTVKG

SEQ ID NO: 28 - protein, 11 aa, synthetic construct
EYYSYDEGFAY

SEQ ID NO: 29 - protein, 12 aa, synthetic construct
SVSDLIPSQYLH

SEQ ID NO: 30 - protein, 7 aa, synthetic construct
RTSNLAS

SEQ ID NO: 31 - protein, 9 aa, synthetic construct
QQGVDVPFT

SEQ ID NO: 32 - protein, 11 aa, synthetic construct
EYYSYDEGFAS

SEQ ID NO: 33 - protein, 7 aa, synthetic construct
DASNLAS

SEQ ID NO: 34 - protein, 5 aa, synthetic construct
HYNMD

SEQ ID NO: 35 - protein, 17 aa, synthetic construct
TIYPGNADTSYNQKFKG

SEQ ID NO: 36 - protein, 8 aa, synthetic construct
GDLYALDY

SEQ ID NO: 37 - protein, 11 aa, synthetic construct
KASQSVYRDVA

SEQ ID NO: 38 - protein, 7 aa, synthetic construct
SASNRYT

SEQ ID NO: 39 - protein, 9 aa, synthetic construct
QHDYSSPYT

SEQ ID NO: 40 - protein, 11 aa, synthetic construct
EYSSYDEGFAY

SEQ ID NO: 41 - protein, 5 aa, synthetic construct
TYNMD

SEQ ID NO: 42 - protein, 17 aa, synthetic construct
TIYPGNGDTSYNQKFKG

SEQ ID NO: 43 - protein, 11 aa, synthetic construct
KASQSVSNDVA

SEQ ID NO: 44 - protein, 5 aa, synthetic construct
HYDMD